European Patent Application EP 4 141 031 A1, published March 1, 2023. Title: ANTIBODY BINDING WITH SPECIFIC EPITOPE IN HUMAN IL-4Rα AND APPLICATIONS OF ANTIBODY. Applicant: SUZHOU CONNECT BIOPHARMACEUTICALS, LTD. The sequence listing filed with the application follows.

SEQUENCE LISTING (72 sequences)

SEQ ID NO: 1 - protein, 232 aa, Homo sapiens
MGWLCSGLLFPVSCLVLLQVASSGNMKVLQEPTCVSDYMSISTCEWKMNGPTNCSTELRLLYQLVFLLSEAHTCIPENNGGAGCVCHLLMDDVVSADNYTLDLWAGQQLLWKGSFKPSEHVKPRAPGNLTVHTNVSDTLLLTWSNPYPPDNYLYNHLTYAVNIWSENDPADFRIYNVTYLEPSLRIAASTLKSGISYRARVRAWAQCYNTTWSEWSPSTKWHNSYREPFEQH

SEQ ID NO: 2 - protein, 232 aa, Macaca fascicularis
MGWLCSGLLFPVSCLVLLQVASSGSMKVLQEPACVSDYMSISTCEWKMGGPTNCSAELRLLYQLVFQSSETHTCVPENNGGVGCVCHLLMDDVVSMDNYTLDLWAGQQLLWKGSFKPSEHVKPRAPGNLTVHTNVSDTVLLTWSNPYPPDNYLYNDLTYAVNIWSENDPAYSRIHNVTYLKPTLRIPASTLKSGISYRARVRAWAQHYNTTWSEWSPSTKWYNSYREPFEQR

SEQ ID NO: 3 - protein, 118 aa, artificial sequence
  Y0188-1, VH
EVQLVESGGGLVQPKGSLKLSCAASGFTFNTYGMHWVRQAPGKGLEWVAHIRSKSSNYATYYADSVKDRFTISRDDSQSMLYLQMNNLKTEDTAMYYCVRWFRAMDYWGQGTSVTVSS

SEQ ID NO: 4 - protein, 107 aa, artificial sequence
  Y0188-1, VL
DIVMTQSHKFMSTSVGDRVSITCKASQDVSTAVAWYQEKPGQSPKLLIYWASTRHTGVPDRFTGSGSGTDYTLTISSVQAEDLALYYCQQHYSTPLTFGAGTKLELK

SEQ ID NO: 5 - protein, 120 aa, artificial sequence
  Y0188-2, VH
EVQLIESGGGLVQPKGSLKLSCAASGFTFNMYAMDWVRQAPGKGLEWVARIRSKGSNFETNYADSVKDRFTISRDDSQSMVYLQMINLKTEDTAMYYCVRHRGGAWFAYWGQGTLVSVSA

SEQ ID NO: 6 - protein, 111 aa, artificial sequence
  Y0188-2, VL
DIVVTQSPASLAVSLGQRATISCRASKSVSTSGYSYMHWYQQKPGQPPKLLIYLASNLESGVPARFSGSGSGTDFTLNIHPVEEEDVAIYYCQHSRELPLTFGAGTKLELK

SEQ ID NO: 7 - protein, 121 aa, artificial sequence
  Y0188-3, VH
QVQLVETGGGLVRPGNSLKLSCVTSGFTFSNYRMHWLRQPPGKRLEWIAVITVKSNNYGANYAESVKGRFAISRDDSKSSVYLEMNRLREEDTATYFCSRERAYGNPFDYWGQGTTLTVSS

SEQ ID NO: 8 - protein, 107 aa, artificial sequence
  Y0188-3, VL
DIQMTQSPSSLSASLGERVSLTCRASQEISGYLSWLQQKPDGTIKRLIYAASTLDSGVPKRFSGSRSGSDYSLTISSLESEDFADYYCLQYGSYPYTFGGGTKLEIK

SEQ ID NO: 9 - protein, 118 aa, artificial sequence
  Y0188-4, VH
EVQLVESGGGLVQPKGSLKLSCAASGFTFNMYAMNWVRQAPGQGLEWVARIRSKSNNYATYYADSVKDRFIISRDDSESMVYLQMSNLRAADTAMYYCVRHLRAMDYWGQGTSVTVSS

SEQ ID NO: 10 - protein, 111 aa, artificial sequence
  Y0188-4, VL
DIVLTQSPASLTVSLGQRATISCRASKSVSTSGYSYMHWYQQKPGQPPKLLIYLASNLESGVPARFSGSGSGTDFTLNIHPVEEEDAATYYCQHSRELPITFGSGTKLEIK

SEQ ID NO: 11 - protein, 118 aa, artificial sequence
  Y0188-6, VH
EVQLVESGGGLVQPKGSLKLSCAASGFSFNMYAMNWVRQAPGKGLEWVARIRTKSNHYSTYYADSVKDRFTISRDDSASMFYLQMNNLKTEDTAMYFCVRHLRAMDYWGQGTSVTVSS

SEQ ID NO: 12 - protein, 111 aa, artificial sequence
  Y0188-6, VL
DIVLTQSPASLVVSLGQRATISCRASQSVSTSGYSYMHWYQQKPGQPPKLLIYLASNVQSGVPARFSGSGSGTDFTLNIHPVEEEDVATYYCHHNRDLPFTFGSGTKLEIK

SEQ ID NO: 13 - protein, 120 aa, artificial sequence
  Y0188-8, VH
EVQLIESGGGLVQPKGSLKLSCAASGFTFNMYAMDWVRQAPGKGLEWVARIRSKGSNFETNYADSVKDRFTISRDDSQSMVYLQMNNLKTEDTAMYYCVRHRGGAWFAYWGQGTLVTVSA

SEQ ID NO: 14 - protein, 111 aa, artificial sequence; identical to SEQ ID NO: 6
  Y0188-8, VL

SEQ ID NO: 15 - protein, 118 aa, artificial sequence
  Y0188-9, VH
EVQLVESGGGLVRPKGSLKLSCAASGFSFNTYAMNWVRQAPGKGLEWIVWIRSKSHNYATYYADSVKDRFTISRDDSESMLYLQMNNLKTEDTAMYYCVRHLRAMDYWGQGTSVTVSS

SEQ ID NO: 16 - protein, 111 aa, artificial sequence
  Y0188-9, VL
DIVLTQSPASLAVSLGQRATISCRASKSVSASGYSYMHWYQQKPGQPPKLLIYLASNLQSGVPARFSGSGSGTDFTLNIHPVEEEDAATYYCQHSRELPPTFGGGTKLEIK

SEQ ID NO: 17 - protein, 118 aa, artificial sequence
  Y0188-10, VH
EVRLVESGGGLVQPKGSLKLSCEASGFSFNMYAMNWVRQAPGKGLEWITHIRSKSNNYATYYADSVKDRFIISRDDSESMVYLQMNNLKTEDTAMYYCVRLLRALDYWGQGTSVTVSS

SEQ ID NO: 18 - protein, 111 aa, artificial sequence
  Y0188-10, VL
DIVLTQSPASLAVFLGQRATISCRASKSVSTSGYSYMHWYQQKAGQPPKLLIYLASNLESGVPARFSGSGSGTDFTLNIHPVEEEDAATYYCHHSRELPITFGSGTKLEMK

SEQ ID NO: 19 - protein, 118 aa, artificial sequence
  Y0188-14, VH
EVQLVESGGGLVQPKGSLKLSCAASGFTFNMYGMHWVRQAPGKGLEWVAHIRSKSSNYATYYADSVKDRLTISRDDSQSMLYLQMNNLKTEDTAMYYCVRWFRAMDYWGQGTSVTVSS

SEQ ID NO: 20 - protein, 107 aa, artificial sequence; identical to SEQ ID NO: 4
  Y0188-14, VL

SEQ ID NO: 21 - protein, 118 aa, artificial sequence
  HV3-15-14H, VH
EVQLVESGGGLVKPGGSLRLSCAASGFTFSMYGMHWVRQAPGKGLEWVGHIRSKSSNYATYYADSVKDRFTISRDDSKNTLYLQMNSLKTEDTAVYYCTTWFRAMDYWGQGTLVTVSS

SEQ ID NO: 22 - protein, 118 aa, artificial sequence
  HV3-48-14H, VH
EVQLVESGGGLVQPGGSLRLSCAASGFTFSMYGMHWVRQAPGKGLEWVSHIRSKSSNYATYYADSVKDRFTISRDNAKNSLYLQMNSLRAEDTAVYYCARWFRAMDYWGQGTLVTVSS

SEQ ID NO: 23 - protein, 118 aa, artificial sequence
  HV3-73*2-14H, VH
EVQLVESGGGLVQPGGSLKLSCAASGFTFSMYGMHWVRQASGKGLEWVGHIRSKSSNYATYYADSVKDRFTISRDDSKNTAYLQMNSLKTEDTAVYYCTRWFRAMDYWGQGTLVTVSS

SEQ ID NO: 24 - protein, 118 aa, artificial sequence
  HV3-72-14H, VH
EVQLVESGGGLVQPGGSLRLSCAASGFTFSMYGMHWVRQAPGKGLEWVGHIRSKSSNYATYYADSVKDRFTISRDDSKNSLYLQMNSLKTEDTAVYYCARWFRAMDYWGQGTLVTVSS

SEQ ID NO: 25 - protein, 118 aa, artificial sequence; identical to SEQ ID NO: 22
  201-14H, VH

SEQ ID NO: 26 - protein, 118 aa, artificial sequence
  162-14H, VH
EVQLVESGGGLEQPGGSLRLSCAGSGFTFRMYGMHWVRQAPGKGLEWVSHIRSKSSNYATYYADSVKDRFTISRDNSKNTLYLQMNSLRAEDTAVYYCAKWFRAMDYWGQGTTVTVSS

SEQ ID NO: 27 - protein, 118 aa, artificial sequence
  VH73-14H, VH
EVQLVESGGGLVQPGGSLKLSCAASGFTFSMYGMHWVRQASGKGLEWVGHIRSKSSNYATYYADSVKDRFTISRDDSKNTAYLQMNSLKTEDTAVYYCTRWFRAMDYWGQGTTVTVSS

SEQ ID NO: 28 - protein, 107 aa, artificial sequence
  Y01-14L, VL
EIVLTQSPGTLSLSPGERATLSCKASQDVSTAVAWYQQKPGQAPRLLIYWASTRHTGIPDRFSGSGSGTDFTLTISRLEPEDFAVYYCQQHYSTPLTFGQGTKVEIK

SEQ ID NO: 29 - protein, 107 aa, artificial sequence
  164-14L, VL
DIVMTQSPLSLPVTPGEPASISCKASQDVSTAVAWYLQKSGQSPQLLIYWASTRHTGVPDRFSGSGSGTDFTLKISRVEAEDVGFYYCQQHYSTPLTFGQGTKLEIK

SEQ ID NO: 30 - protein, 107 aa, artificial sequence
  KV4-14L, VL
DIVMTQSPDSLAVSLGERATINCKASQDVSTAVAWYQQKPGQPPKLLIYWASTRHTGVPDRFSGSGSGTDFTLTISSLQAEDVAVYYCQQHYSTPLTFGGGTKVEIK

SEQ ID NO: 31 - protein, 107 aa, artificial sequence
  KV1-27-14L, VL
DIQMTQSPSSLSASVGDRVTITCKASQDVSTAVAWYQQKPGKVPKLLIYWASTRHTGVPSRFSGSGSGTDFTLTISSLQPEDVATYYCQQHYSTPLTFGGGTKVEIK

SEQ ID NO: 32 - protein, 107 aa, artificial sequence
  KV1-9-14L, VL
DIQLTQSPSFLSASVGDRVTITCKASQDVSTAVAWYQQKPGKAPKLLIYWASTRHTGVPSRFSGSGSGTEFTLTISSLQPEDFATYYCQQHYSTPLTFGGGTKVEIK

SEQ ID NO: 33 - protein, 107 aa, artificial sequence
  KV1-NL1-14L, VL
DIQMTQSPSSLSASVGDRVTITCKASQDVSTAVAWYQQKPGKAPKLLLYWASTRHTGVPSRFSGSGSGTDYTLTISSLQPEDFATYYCQQHYSTPLTFGGGTKVEIK

SEQ ID NO: 34 - protein, 107 aa, artificial sequence
  KV1D-43-14L, VL
AIRMTQSPFSLSASVGDRVTITCKASQDVSTAVAWYQQKPAKAPKLFIYWASTRHTGVPSRFSGSGSGTDYTLTISSLQPEDFATYYCQQHYSTPLTFGGGTKVEIK

SEQ ID NO: 35 - protein, 5 aa, artificial sequence
  HCDR1
TYGMH

SEQ ID NO: 36 - protein, 19 aa, artificial sequence
  HCDR2
HIRSKSSNYATYYADSVKD

SEQ ID NO: 37 - protein, 7 aa, artificial sequence
  HCDR3
WFRAMDY

SEQ ID NO: 38 - protein, 5 aa, artificial sequence
  HCDR1
MYAMD

SEQ ID NO: 39 - protein, 19 aa, artificial sequence
  HCDR2
RIRSKGSNFETNYADSVKD

SEQ ID NO: 40 - protein, 9 aa, artificial sequence
  HCDR3
HRGGAWFAY

SEQ ID NO: 41 - protein, 5 aa, artificial sequence
  HCDR1
NYRMH

SEQ ID NO: 42 - protein, 19 aa, artificial sequence
  HCDR2
VITVKSNNYGANYAESVKG

SEQ ID NO: 43 - protein, 10 aa, artificial sequence
  HCDR3
ERAYGNPFDY

SEQ ID NO: 44 - protein, 5 aa, artificial sequence
  HCDR1
MYAMN

SEQ ID NO: 45 - protein, 19 aa, artificial sequence
  HCDR2
RIRSKSNNYATYYADSVKD

SEQ ID NO: 46 - protein, 7 aa, artificial sequence
  HCDR3
HLRAMDY

SEQ ID NO: 47 - protein, 19 aa, artificial sequence
  HCDR2
RIRTKSNHYSTYYADSVKD

SEQ ID NO: 48 - protein, 5 aa, artificial sequence
  HCDR1
TYAMN

SEQ ID NO: 49 - protein, 19 aa, artificial sequence
  HCDR2
WIRSKSHNYATYYADSVKD

SEQ ID NO: 50 - protein, 19 aa, artificial sequence
  HCDR2
HIRSKSNNYATYYADSVKD

SEQ ID NO: 51 - protein, 7 aa, artificial sequence
  HCDR3
LLRALDY

SEQ ID NO: 52 - protein, 5 aa, artificial sequence
  HCDR1
MYGMH

SEQ ID NO: 53 - protein, 11 aa, artificial sequence
  LCDR1
KASQDVSTAVA

SEQ ID NO: 54 - protein, 7 aa, artificial sequence
  LCDR2
WASTRHT

SEQ ID NO: 55 - protein, 9 aa, artificial sequence
  LCDR3
QQHYSTPLT

SEQ ID NO: 56 - protein, 15 aa, artificial sequence
  LCDR1
RASKSVSTSGYSYMH

SEQ ID NO: 57 - protein, 7 aa, artificial sequence
  LCDR2
LASNLES

SEQ ID NO: 58 - protein, 9 aa, artificial sequence
  LCDR3
QHSRELPLT

SEQ ID NO: 59 - protein, 11 aa, artificial sequence
  LCDR1
RASQEISGYLS

SEQ ID NO: 60 - protein, 7 aa, artificial sequence
  LCDR2
AASTLDS

SEQ ID NO: 61 - protein, 9 aa, artificial sequence
  LCDR3
LQYGSYPYT

SEQ ID NO: 62 - protein, 9 aa, artificial sequence
  LCDR3
QHSRELPIT

SEQ ID NO: 63 - protein, 15 aa, artificial sequence
  LCDR1
RASQSVSTSGYSYMH

SEQ ID NO: 64 - protein, 7 aa, artificial sequence
  LCDR2
LASNVQS

SEQ ID NO: 65 - protein, 9 aa, artificial sequence
  LCDR3
HHNRDLPFT

SEQ ID NO: 66 - protein, 15 aa, artificial sequence
  LCDR1
RASKSVSASGYSYMH

SEQ ID NO: 67 - protein, 7 aa, artificial sequence
  LCDR2
LASNLQS

SEQ ID NO: 68 - protein, 9 aa, artificial sequence
  LCDR3
QHSRELPPT

SEQ ID NO: 69 - protein, 9 aa, artificial sequence
  LCDR3
HHSRELPIT

SEQ ID NO: 70 - DNA, 993 bp, Homo sapiens
gctagcaccaagggcccatcggtcttccccctggcaccctcctccaagagcacctctgggggcacagcggccctgggctgcctggtcaaggactacttccccgaaccggtgacggtgtcgtggaactcaggcgccctgaccagcggcgtgcacaccttcccggctgtcctacagtcctcaggactctactccctcagcagcgtggtgaccgtgccctccagcagcttgggcacccagacctacatctgcaacgtgaatcacaagcccagcaacaccaaggtggacaagaaagttgagcccaaatcttgtgacaaaactcacacatgcccaccgtgcccagcacctgaactcctggggggaccgtcagtcttcctcttccccccaaaacccaaggacaccctcatgatctcccggacccctgaggtcacatgcgtggtggtggacgtgagccacgaagaccctgaggtcaagttcaactggtacgtggacggcgtggaggtgcataatgccaagacaaagccgcgggaggagcagtacaacagcacgtaccgtgtggtcagcgtcctcaccgtcctgcaccaggactggctgaatggcaaggagtacaagtgcaaggtctccaacaaagccctcccagcccccatcgagaaaaccatctccaaagccaaagggcagccccgagaaccacaggtgtacaccctgcccccatcccgggaggagatgaccaagaaccaggtcagcctgacctgcctggtcaaaggcttctatcccagcgacatcgccgtggagtgggagagcaatgggcagccggagaacaactacaagaccacgcctcccgtgctggactccgacggctccttcttcctctacagcaagctcaccgtggacaagagcaggtggcagcaggggaacgtcttctcatgctccgtgatgcacgaggctctgcacaaccactacacgcagaagagcctctccctgtctccgggtaaatga

SEQ ID NO: 71 - DNA, 995 bp, Homo sapiens
gctagcaccaagggcccatcggtcttccccctggcgccctgctccaggagcacctccgagagcacagccgccctgggctgcctggtcaaggactacttccccgaaccggtgacggtgtcgtggaactcaggcgccctgaccagcggcgtgcacaccttcccggctgtcctacagtcctcaggactctactccctcagcagcgtggtgaccgtgccctccagcagcttgggcacgaagacctacacctgcaacgtagatcacaagcccagcaacaccaaggtggacaagagagttgagtccaaatatggtcccccatgcccatcatgcccagcacctgagttcctggggggaccatcagtcttcctgttccccccaaaacccaaggacactctcatgatctcccggacccctgaggtcacgtgcgtggtggtggacgtgagccaggaagaccccgaggtccagttcaactggtacgtggatggcgtggaggtgcataatgccaagacaaagccgcgggaggagcagttcaacagcacgtaccgtgtggtcagcgtcctcaccgtcctgcaccaggactggctgaacggcaaggagtacaagtgcaaggtctccaacaaaggcctcccgtcctccatcgagaaaaccatctccaaagccaaagggcagccccgagagccacaggtgtacaccctgcccccatcccaggaggagatgaccaagaaccaggtcagcctgacctgcctggtcaaaggcttctaccccagcgacatcgccgtggagtgggagagcaatgggcagccggagaacaactacaagaccacgcctcccgtgctggactccgacggctccttcttcctctacagcaggctcaccgtggacaagagcaggtggcaggaggggaatgtcttctcatgctccgtgatgcatgaggctctgcacaaccactacacacagaagagcctctccctgtctccgggtaaatgagttctagctgg

SEQ ID NO: 72 - DNA, 327 bp, Homo sapiens
acggtggctgcaccatctgtcttcatcttcccgccatctgatgagcagttgaaatctggaactgcctctgttgtgtgcctgctgaataacttctatcccagagaggccaaagtacagtggaaggtggataacgccctccaatcgggtaactcccaggagagtgtcacagagcaggacagcaaggacagcacctacagcctcagcagcaccctgacgctgagcaaagcagactacgagaaacacaaagtctacgcctgcgaagtcacccatcagggcctgagctcgcccgtcacaaagagcttcaacaggggagagtgttagagggag